European Patent Specification EP 3 634 443 B1, published September 18, 2024. Title: MICROBIOME BIOMARKERS OF IMMUNOTHERAPY RESPONSIVENESS: DIAGNOSTIC, PROGNOSTIC AND THERAPEUTIC USES THEREOF. Applicant: THE UNIVERSITY OF CHICAGO. The sequence listing filed with the application follows.

SEQUENCE LISTING (34 sequences)

SEQ ID NO: 1 - DNA, 20 bp, Artificial sequence
  Synthetic
cagcacgtgaaggtggggac

SEQ ID NO: 2 - DNA, 20 bp, Artificial sequence
  Synthetic
ccttgcggttggcttcagat

SEQ ID NO: 3 - DNA, 23 bp, Artificial sequence
  Synthetic
aagggagcgtagatggatgttta

SEQ ID NO: 4 - DNA, 20 bp, Artificial sequence
  Synthetic
cgagcctcaatgtcagttgc

SEQ ID NO: 5 - DNA, 31 bp, Artificial sequence
  Synthetic
cctgcctcaactgcactcaagatatccagta

SEQ ID NO: 6 - DNA, 23 bp, Artificial sequence
  Synthetic
ctccgccgctgatccggaagtcg

SEQ ID NO: 7 - DNA, 25 bp, Artificial sequence
  Synthetic
aaccaactcggcgatgtggacgaca

SEQ ID NO: 8 - DNA, 20 bp, Artificial sequence
  Synthetic
ttccagttgatcgcatggtc

SEQ ID NO: 9 - DNA, 18 bp, Artificial sequence
  Synthetic
  misc_feature (3)..(3): n is g or c
tcncgcttgctccccgat

SEQ ID NO: 10 - DNA, 16 bp, Artificial sequence
  Synthetic
cccgacgggaggggat

SEQ ID NO: 11 - DNA, 21 bp, Artificial sequence
  Synthetic
cttctgcaggtacagtcttga

SEQ ID NO: 12 - DNA, 26 bp, Artificial sequence
  Synthetic
cgagaagagctgcaaaatgctttagc

SEQ ID NO: 13 - DNA, 19 bp, Artificial sequence
  Synthetic
gcgcgcttcaattccttgt

SEQ ID NO: 14 - DNA, 17 bp, Artificial sequence
  Synthetic
cccttcagtgccgcagt

SEQ ID NO: 15 - DNA, 18 bp, Artificial sequence
  Synthetic
gtcgcaggatgtcaagac

SEQ ID NO: 16 - DNA, 24 bp, Artificial sequence
  Synthetic
gcgtggcggtagatctaagtcata

SEQ ID NO: 17 - DNA, 21 bp, Artificial sequence
  Synthetic
ttcagctccgccacaaaggta

SEQ ID NO: 18 - DNA, 21 bp, Artificial sequence
  Synthetic
caccgaatgcttgcaytcacc

SEQ ID NO: 19 - DNA, 19 bp, Artificial sequence
  Synthetic
gccgcgggtccatccaaaa

SEQ ID NO: 20 - DNA, 21 bp, Artificial sequence
  Synthetic
tgcctatcagagggggataac

SEQ ID NO: 21 - DNA, 21 bp, Artificial sequence
  Synthetic
gcaaatattcccatgcgggat

SEQ ID NO: 22 - DNA, 28 bp, Artificial sequence
  Synthetic
cgaaagtcggactaataccgcatgaagc

SEQ ID NO: 23 - DNA, 19 bp, Artificial sequence
  Synthetic
agggtgcgtaggtggtgat

SEQ ID NO: 24 - DNA, 18 bp, Artificial sequence
  Synthetic
ttcaccgctacaccacgc

SEQ ID NO: 25 - DNA, 27 bp, Artificial sequence
  Synthetic
ttacttgagtgtgtttgaggtaggcgg

SEQ ID NO: 26 - DNA, 20 bp, Artificial sequence
  Synthetic
ttcgcagctcagtctatcgc

SEQ ID NO: 27 - DNA, 20 bp, Artificial sequence
  Synthetic
gcaatccccgggaagtcatt

SEQ ID NO: 28 - DNA, 18 bp, Artificial sequence
  Synthetic
gcagatttggtctgtttc

SEQ ID NO: 29 - DNA, 19 bp, Artificial sequence
  Synthetic
cggtattagcaaccatttc

SEQ ID NO: 30 - DNA, 24 bp, Artificial sequence
  Synthetic
ctgtataaggcaggttacccacgc

SEQ ID NO: 31 - DNA, 18 bp, Artificial sequence
  Synthetic
  misc_feature (2)..(2): n is c or t
ancaacctgcccttcaga

SEQ ID NO: 32 - DNA, 20 bp, Artificial sequence
  Synthetic
cgtcccgattaacagagctt

SEQ ID NO: 33 - DNA, 20 bp, Artificial sequence
  Synthetic
agagtttgatcctggctcag

SEQ ID NO: 34 - DNA, 18 bp, Artificial sequence
  Synthetic
tgctgcctcccgtaggag